European Patent Application EP 4 759 826 A1, published June 17, 2026. Title: peptide fragment and use thereof. Applicant: TOAGOSEI CO., LTD. The sequence listing filed with the application follows.

SEQUENCE LISTING (4 sequences)

SEQ ID NO: 1 - protein, 16 aa, synthetic construct
KKRTLRKYLIQFRKKR

SEQ ID NO: 2 - protein, 16 aa, synthetic construct
KKRTLRKFQILYRKKR

SEQ ID NO: 3 - protein, 16 aa, synthetic construct
KKRTLRKYQFLIRKKR

SEQ ID NO: 4 - protein, 16 aa, synthetic construct
KKRTLRKILFQYRKKR